European Patent Application EP 4 129 285 A1, published February 8, 2023. Title: Compounds for use in regulating follicle maturation. Applicant: Aarhus Universitet. Application EP. The sequence listing filed with the application follows.

SEQUENCE LISTING (1 sequence)

SEQ ID NO: 1 - protein, 126 aa, Homo sapiens
MSIEEAVPAVCKTRTVIYEIPRSQVDPTSANFLIWPPCVEVKRCTGCCNTSSVKCQPSRVHHRSVKVAKVEYVRKKPKLKEVQVRLEEHLECACATSNLNPDHREEETGRRRESGKNRKRKRLKPT